European Patent Specification EP 3 464 344 B1, published December 13, 2023. Title: CELL. Applicant: UCL Business PLC. The sequence listing filed with the application follows.

SEQUENCE LISTING (61 sequences)

SEQ ID NO: 1 - protein, 346 aa, Homo sapiens
MYNGSCCRIEGDTISQVMPPLLIVAFVLGALGNGVALCGFCFHMKTWKPSTVYLFNLAVADFLLMICLPFRTDYYLRRRHWAFGDIPCRVGLFTLAMNRAGSIVFLTVVAADRYFKVVHPHHAVNTISTRVAAGIVCTLWALVILGTVYLLLENHLCVQETAVSCESFIMESANGWHDIMFQLEFFMPLGIILFCSFKIVWSLRRRQQLARQARMKKATRFIMVVAIVFITCYLPSVSARLYFLWTVPSSACDPSVHGALHITLSFTYMNSMLDPLVYYFSSPSFPKFYNKLKICSLKPKQPGHSKTQRPEEMPISNLGRRSCISVANSFQSQSDGQWDPHIVEWH

SEQ ID NO: 2 - protein, 362 aa, Homo sapiens
MGNHTWEGCHVDSRVDHLFPPSLYIFVIGVGLPTNCLALWAAYRQVQQRNELGVYLMNLSIADLLYICTLPLWVDYFLHHDNWIHGPGSCKLFGFIFYTNIYISIAFLCCISVDRYLAVAHPLRFARLRRVKTAVAVSSVVWATELGANSAPLFHDELFRDRYNHTFCFEKFPMEGWVAWMNLYRVFVGFLFPWALMLLSYRGILRAVRGSVSTERQEKAKIKRLALSLIAIVLVCFAPYHVLLLSRSAIYLGRPWDCGFEERVFSAYHSSLAFTSLNCVADPILYCLVNEGARSDVAKALHNLLRFLASDKPQEMANASLTLETPLTSKRNSTAKAMTGSWAATPPSQGDQVQLKMLPPAQ

SEQ ID NO: 3 - protein, 365 aa, Homo sapiens
MGNITADNSSMSCTIDHTIHQTLAPVVYVTVLVVGFPANCLSLYFGYLQIKARNELGVYLCNLTVADLFYICSLPFWLQYVLQHDNWSHGDLSCQVCGILLYENIYISVGFLCCISVDRYLAVAHPFRFHQFRTLKAAVGVSVVIWAKELLTSIYFLMHEEVIEDENQHRVCFEHYPIQAWQRAINYYRFLVGFLFPICLLLASYQGILRAVRRSHGTQKSRKDQIQRLVLSTVVIFLACFLPYHVLLLVRSVWEASCDFAKGVFNAYHFSLLLTSFNCVADPVLYCFVSETTHRDLARLRGACLAFLTCSRTGRAREAYPLGAPEASGKSGAQGEEPELLTKLHPAFQTPNSPGSGGFPTGRLA

SEQ ID NO: 4 - protein, 337 aa, Homo sapiens
MNSTCIEEQHDLDHYLFPIVYIFVIIVSIPANIGSLCVSFLQAKKESELGIYLFSLSLSDLLYALTLPLWIDYTWNKDNWTFSPALCKGSAFLMYMNFYSSTAFLTCIAVDRYLAVVYPLKFFFLRTRRFALMVSLSIWILETIFNAVMLWEDETVVEYCDAEKSNFTLCYDKYPLEKWQINLNLFRTCTGYAIPLVTILICNRKVYQAVRHNKATENKEKKRIIKLLVSITVTFVLCFTPFHVMLLIRCILEHAVNFEDHSNSGKRTYTMYRITVALTSLNCVADPILYCFVTETGRYDMWNILKFCTGRCNTSQRQRKRILSVSTKDTMELEVLE

SEQ ID NO: 5 - protein, 147 aa, Artificial Sequence
  GAL4 DNA binding domain
MRKLLSSIEQACDICRLKKLKCSKEKPKCAKCLKNNWECRYSPKTKRSPLTRAHLTEVESRLERLEQLFLLIFPREDLDMILKMDSLQDIKALLTGLFVQDNVNKDAVTDRLASVETDMPLTLRQHRISATSSSEESSNKGQRQLTV

SEQ ID NO: 6 - DNA, 17 bp, Artificial Sequence
  upstream activating sequence (UAS)
  misc_feature (4)..(14): n is a, c, g, or t
cggnnnnnnnnnnnccg

SEQ ID NO: 7 - protein, 78 aa, Artificial Sequence
  transcriptional activator VP16
APPTDVSLGDELHLDGEDVAMAHADALDDFDLDMLGDGDSPGPGFTPHDSAPYGALDMADFEFEQMFTDALGIDEYGG

SEQ ID NO: 8 - protein, 551 aa, Artificial Sequence
  transcriptional activator p65
MDELFPLIFPAEPAQASGPYVEIIEQPKQRGMRFRYKCEGRSAGSIPGERSTDTTKTHPTIKINGYTGPGTVRISLVTKDPPHRPHPHELVGKDCRDGFYEAELCPDRCIHSFQNLGIQCVKKRDLEQAISQRIQTNNNPFQVPIEEQRGDYDLNAVRLCFQVTVRDPSGRPLRLPPVLSHPIFDNRAPNTAELKICRVNRNSGSCLGGDEIFLLCDKVQKEDIEVYFTGPGWEARGSFSQADVHRQVAIVFRTPPYADPSLQAPVRVSMQLRRPSDRELSEPMEFQYLPDTDDRHRIEEKRKRTYETFKSIMKKSPFSGPTDPRPPPRRIAVPSRSSASVPKPAPQPYPFTSSLSTINYDEFPTMVFPSGQISQASALAPAPPQVLPQAPAPAPAPAMVSALAQAPAPVPVLAPGPPQAVAPPAPKPTQAGEGTLSEALLQLQFDDEDLGALLGNSTDPAVFTDLASVDNSEFQQLLNQGIPVAPHTTEPMLMEYPEAITRLVTGAQRPPDPAPAPLGAPGLPNGLLSGDEDFSSIADMDFSALLSQISS

SEQ ID NO: 9 - protein, 188 aa, Artificial Sequence
  transcriptional repressor SSX3
MNGDDTFARRPTVGAQIPEKIQKAFDDIAKYFSKEEWEKMKVSEKIVYVYMKRKYEAMTKLGFKAILPSFMRNKRVTDFQGNDFDNDPNRGNQVQRPQMTFGRLQGIFPKIMPKKPAEEGNVSKEVPEASGPQNDGKQLCPPGKPTTSEKINMISGPKRGEHAWTHRLRERKQLVIYEEISDPEEDDE

SEQ ID NO: 10 - protein, 962 aa, Artificial Sequence
  transcriptional repressor V-Erb-A
METVIKVISSAPVVAMPVVIKTEGPAWTPLEPEDTRWLDGKHKRKSSQCLVKSSMSGYIPSCLDKDEQCVVCGDKPTGYHYRCITCEGCKSFFRRTIQKNLHPTYSCTYDGCCVIDKITRNQCQLCRFKKCISVGMAMDLVLDDSKRVAKRKLIEENRERRRKEEMIKSLQHRPSPSAEEWELIHVVTEAHRSTNAQGSHWKQRRKFLLEDIGQSPMASMLDGDKVDLEAFTEFTKIITPAITRVVDFAKNLPMFSELPCEDQIILLKGCCMEIMSLRAAVRYDPESETLTLSGEMAVKREQLKNGGLGVVSDAIFDLGKSLSAFNLDDTEVALLQAVLLMSSDRTGLICVDKIEKCQESYLLAFEHYINYRKHNIPHFWSKLLMKVADLRMIGAYHASRFLHMKVECPTELSPQEVGPDHCMKCAHFIDGPHCVKACPAGVLGENDTLVWKYADANAVCQLCHPNCTRGCKGPGLEGCPNGSKTPSIAAGVVGGLLCLVVVGLGIGLYLRRRHIVRKRTLRRLLQERELVEPLTPSGEAPNQAHLRILKETEFKKVKVLGFGAFGTVYKGLWIPEGEKVTIPVAIKELREATSPKANKEILDEAYVMASVDNPHVCRLLGICLTSTVQLITQLMPYGCLLDYIREHKDNIGSQYLLNWCVQIAKGMNYLEERHMVHRDLAARNVLVKTPQHVKITDFGLAKQLGADEKEYHAEGGKVPIKWMALESILHRIYTHQSDVWSYGVTVWELMTFGSKPYDGIPASEISSVLEKGERLPQPPICTIDVYMIMVKCWMSGADSRPKFRELIAEFSKMARDPPRYLVIQGDERMHLPSPTDSKFYRTLMEEEDMEDIVDADEYLVPHQGFFNSPSTSRTPLLSSLSATSNNSATKCIDRNGGHPVREDGFLPAPEYVNQLMPKKPSTAMVQNQIYNYISLTAISKLPMDSRYQNSHSTAVDNPEYLE

SEQ ID NO: 11 - protein, 205 aa, Artificial Sequence
  transcriptional repressor Tetracycline repressor (TetR)
RLDKSKVINSALELLNEVGIEGLTTRKLAQKLGVEQPTLYWHVKNKRALLDALAIEMLDRHHTHFCPLEGESWQDFLRNNAKSFRCALLSHRDGAKVHLGTRPTEKQYETLENQLAFLCQQGFSLENALYALSAVGHFTLGCVLEDQEHQVAKEERETPTTDSMPPLLRQAIELFDHQGAEPAFLFGLELIICGLEKQLKCESGS

SEQ ID NO: 12 - protein, 20 aa, Artificial Sequence
  TetR DNA binding domain
TTRKLAQKLGVEQPTLYWHV

SEQ ID NO: 13 - DNA, 368 bp, Artificial Sequence
  Tetracycline response element (TRE3GS promoter)
gagtttactccctatcagtgatagagaacgtatgaagagtttactccctatcagtgatagagaacgtatgcagactttactccctatcagtgatagagaacgtataaggagtttactccctatcagtgatagagaacgtatgaccagtttactccctatcagtgatagagaacgtatctacagtttactccctatcagtgatagagaacgtatatccagtttactccctatcagtgatagagaacgtataagctttgcttatgtaaaccagggcgcctataaaagagtgctgattttttgagtaaacttcaattccacaacacttttgtcttataccaactttccgtaccacttcctaccctcgtaaa

SEQ ID NO: 14 - protein, 7 aa, Artificial Sequence
  SV40 Large T-antigen nuclear localisation signal (NLS)
PKKKRKV

SEQ ID NO: 15 - protein, 20 aa, Artificial Sequence
  nucleoplasmin NLS
AVKRPAATKKAGQAKKKKLD

SEQ ID NO: 16 - protein, 25 aa, Artificial Sequence
  EGL-13 NLS
MSRRRKANPTKLSENAKKLAKEVEN

SEQ ID NO: 17 - protein, 9 aa, Artificial Sequence
  c-Myc NLS
PAAKRVKLD

SEQ ID NO: 18 - protein, 9 aa, Artificial Sequence
  TUS-protein NLS
KLKIKRPVK

SEQ ID NO: 19 - protein, 405 aa, Homo sapiens
MAASGKTSKSEPNHVIFKKISRDKSVTIYLGNRDYIDHVSQVQPVDGVVLVDPDLVKGKKVYVTLTCAFRYGQEDIDVIGLTFRRDLYFSRVQVYPPVGAASTPTKLQESLLKKLGSNTYPFLLTFPDYLPCSVMLQPAPQDSGKSCGVDFEVKAFATDSTDAEEDKIPKKSSVRLLIRKVQHAPLEMGPQPRAEAAWQFFMSDKPLHLAVSLNKEIYFHGEPIPVTVTVTNNTEKTVKKIKAFVEQVANVVLYSSDYYVKPVAMEEAQEKVPPNSTLTKTLTLLPLLANNRERRGIALDGKIKHEDTNLASSTIIKEGIDRTVLGILVSYQIKVKLTVSGFLGELTSSEVATEVPFRLMHPQPEDPAKESYQDANLVFEEFARHNLKDAGEAEEGKRDKNDVDE

SEQ ID NO: 20 - protein, 418 aa, Homo sapiens
MGDKGTRVFKKASPNGKLTVYLGKRDFVDHIDLVDPVDGVVLVDPEYLKERRVYVTLTCAFRYGREDLDVLGLTFRKDLFVANVQSFPPAPEDKKPLTRLQERLIKKLGEHAYPFTFEIPPNLPCSVTLQPGPEDTGKACGVDYEVKAFCAENLEEKIHKRNSVRLVIRKVQYAPERPGPQPTAETTRQFLMSDKPLHLEASLDKEIYYHGEPISVNVHVTNNTNKTVKKIKISVRQYADICLFNTAQYKCPVAMEEADDTVAPSSTFCKVYTLTPFLANNREKRGLALDGKLKHEDTNLASSTLLREGANREILGIIVSYKVKVKLVVSRGGLLGDLASSDVAVELPFTLMHPKPKEEPPHREVPENETPVDTNLIELDTNDDDIVFEDFARQRLKGMKDDKEEEEDGTGSPQLNNR

SEQ ID NO: 21 - protein, 409 aa, Homo sapiens
MGEKPGTRVFKKSSPNCKLTVYLGKRDFVDHLDKVDPVDGVVLVDPDYLKDRKVFVTLTCAFRYGREDLDVLGLSFRKDLFIATYQAFPPVPNPPRPPTRLQDRLLRKLGQHAHPFFFTIPQNLPCSVTLQPGPEDTGKACGVDFEIRAFCAKSLEEKSHKRNSVRLVIRKVQFAPEKPGPQPSAETTRHFLMSDRSLHLEASLDKELYYHGEPLNVNVHVTNNSTKTVKKIKVSVRQYADICLFSTAQYKCPVAQLEQDDQVSPSSTFCKVYTITPLLSDNREKRGLALDGKLKHEDTNLASSTIVKEGANKEVLGILVSYRVKVKLVVSRGGDVSVELPFVLMHPKPHDHIPLPRPQSAAPETDVPVDTNLIEFDTNYATDDDIVFEDFARLRLKGMKDDDYDDQLC

SEQ ID NO: 22 - protein, 388 aa, Homo sapiens
MSKVFKKTSSNGKLSIYLGKRDFVDHVDTVEPIDGVVLVDPEYLKCRKLFVMLTCAFRYGRDDLEVIGLTFRKDLYVQTLQVVPAESSSPQGPLTVLQERLLHKLGDNAYPFTLQMVTNLPCSVTLQPGPEDAGKPCGIDFEVKSFCAENPEETVSKRDYVRLVVRKVQFAPPEAGPGPSAQTIRRFLLSAQPLQLQAWMDREVHYHGEPISVNVSINNCTNKVIKKIKISVDQITDVVLYSLDKYTKTVFIQEFTETVAANSSFSQSFAVTPILAASCQKRGLALDGKLKHEDTNLASSTIIRPGMDKELLGILVSYKVRVNLMVSCGGILGDLTASDVGVELPLVLIHPKPSHEAASSEDIVIEEFTRKGEEESQKAVEAEGDEGS

SEQ ID NO: 23 - protein, 7 aa, Artificial Sequence
  consensus Tobacco Etch Virus (TEV) cleavage site
ENLYFQS

SEQ ID NO: 24 - protein, 240 aa, Artificial Sequence
  TEV protease
SLFKGPRDYNPISSTICHLTNESDGHTTSLYGIGFGPFIITNKHLFRRNNGTLLVQSLHGVFKVKNTTTLQQHLIDGRDMIIIRMPKDFPPFPQKLKFREPQREERICLVTTNFQTKSMSSMVSDTSCTFPSSDGIFWKHWIQTKDGQCGSPLVSTRDGFIVGIHSASNFTNTNNYFTSVPKNFMELLTNQEAQQWVSGWRLNADSVLWGGHKVFMSKPEEPFQPVKEATQLMNELVYSQ

SEQ ID NO: 25 - protein, 4 aa, Artificial Sequence
  basic amino acid furin target sequence
  misc_feature (2)..(2): Xaa can be any naturally occurring amino acid
  MISC_FEATURE (3)..(3): Xaa may be Arg or Lys
RXXR

SEQ ID NO: 26 - protein, 794 aa, Homo sapiens
MELRPWLLWVVAATGTLVLLAADAQGQKVFTNTWAVRIPGGPAVANSVARKHGFLNLGQIFGDYYHFWHRGVTKRSLSPHRPRHSRLQREPQVQWLEQQVAKRRTKRDVYQEPTDPKFPQQWYLSGVTQRDLNVKAAWAQGYTGHGIVVSILDDGIEKNHPDLAGNYDPGASFDVNDQDPDPQPRYTQMNDNRHGTRCAGEVAAVANNGVCGVGVAYNARIGGVRMLDGEVTDAVEARSLGLNPNHIHIYSASWGPEDDGKTVDGPARLAEEAFFRGVSQGRGGLGSIFVWASGNGGREHDSCNCDGYTNSIYTLSISSATQFGNVPWYSEACSSTLATTYSSGNQNEKQIVTTDLRQKCTESHTGTSASAPLAAGIIALTLEANKNLTWRDMQHLVVQTSKPAHLNANDWATNGVGRKVSHSYGYGLLDAGAMVALAQNWTTVAPQRKCIIDILTEPKDIGKRLEVRKTVTACLGEPNHITRLEHAQARLTLSYNRRGDLAIHLVSPMGTRSTLLAARPHDYSADGFNDWAFMTTHSWDEDPSGEWVLEIENTSEANNYGTLTKFTLVLYGTAPEGLPVPPESSGCKTLTSSQACVVCEEGFSLHQKSCVQHCPPGFAPQVLDTHYSTENDVETIRASVCAPCHASCATCQGPALTDCLSCPSHASLDPVEQTCSRQSQSSRESPPQQQPPRLPPEVEAGQRLRAGLLPSHLPEVVAGLSCAFIVLVFVTVFLVLQLRSGFSFRGVKVYTMDRGLISYKGLPPEAWQEECPSDSEEDEGRGERTAFIKDQSAL

SEQ ID NO: 27 - protein, 8 aa, Artificial Sequence
  tobacco vein mottling virus (TVMV) cleavage site
ETVRFQGS

SEQ ID NO: 28 - protein, 241 aa, Artificial Sequence
  TVMV protease
SKALLKGVRDFNPISACVWLLENSSDGHSERLFGIGFGPYIIANQHLFRRNNGELTIKTMHGEFKVKNSTQLQMKPVEGRDIIVIKMAKDFPPFPQKLKFRQPTIKDRVCMVSTNFQQKSVSSLVSESSHIVHKEDTSFWQHWITTKDGQCGSPLVSIIDGNILGIHSLTHTTNGSNYFVEFPEKFVATYLDAADGWCKNWKFNADKISWGSFTLVEDAPEDDFMAKKTVAAIMDDLVRTQ

SEQ ID NO: 29 - protein, 453 aa, Artificial Sequence
  plum pox virus Nia protease
QFWDGFTNSFMQCKLRETDHQCTSDLDVKECGYVAAIVCQAIIPCGKITCLQCAQKYSYMSQQEIRDRFSTVIEQHEKTVMDNYPQFSHVLAFLKRYRELMRVENQNYEALKDITHMIGERKEAPFSHLNKINELIIKGGMMSAQDYMEASNCLRELARYQKNRTENIQSGSIKAFRNKISAKAYVNMQLMCDNQLDTNGNFVWGQREYHAKRFFRNYFDVIDTSEGYRRHIVRENPRGTRKLAIGNLVMSTNLAALRRQLLGEECTNFDVSKECTSKRGENFVYQCCCVTHEDGTPLKSEIISPTKNHLVIGNSGDSKYVDLPKTDKGGMYIAKAGYCYINVFLAMLVNVNESEAKSFTKTVRDTLVPKLGLWPSMMDLATACHFLAVLYPETRNAELPRILVDHESKLFHVVDSYGSLSTGLHILKANTVNQLISFASDTLDSSMKMYLVG

SEQ ID NO: 30 - protein, 21 aa, Artificial Sequence
  signal peptide
MGTSLLCWMALCLLGADHADG

SEQ ID NO: 31 - protein, 21 aa, Artificial Sequence
  signal peptide
MSLPVTALLLPLALLLHAARP

SEQ ID NO: 32 - protein, 20 aa, Artificial Sequence
  signal peptide
MAVPTQVLGLLLLWLTDARC

SEQ ID NO: 33 - protein, 234 aa, Artificial Sequence
  spacer sequence, hinge-CH2CH3 of human IgG1
AEPKSPDKTHTCPPCPAPPVAGPSVFLFPPKPKDTLMIARTPEVTCVVVDVSHEDPEVKFNWYVDGVEVHNAKTKPREEQYNSTYRVVSVLTVLHQDWLNGKEYKCKVSNKALPAPIEKTISKAKGQPREPQVYTLPPSRDELTKNQVSLTCLVKGFYPSDIAVEWESNGQPENNYKTTPPVLDSDGSFFLYSKLTVDKSRWQQGNVFSCSVMHEALHNHYTQKSLSLSPGKKD

SEQ ID NO: 34 - protein, 46 aa, Artificial Sequence
  spacer sequence, human CD8 stalk
TTTPAPRPPTPAPTIASQPLSLRPEACRPAAGGAVHTRGLDFACDI

SEQ ID NO: 35 - protein, 20 aa, Artificial Sequence
  spacer sequence, human IgG1 hinge
AEPKSPDKTHTCPPCPKDPK

SEQ ID NO: 36 - protein, 185 aa, Artificial Sequence
  spacer sequence, CD2 ectodomain
KEITNALETWGALGQDINLDIPSFQMSDDIDDIKWEKTSDKKKIAQFRKEKETFKEKDTYKLFKNGTLKIKHLKTDDQDIYKVSIYDTKGKNVLEKIFDLKIQERVSKPKISWTCINTTLTCEVMNGTDPELNLYQDGKHLKLSQRVITHKWTTSLSAKFKCTAGNKVSKESSVEPVSCPEKGLD

SEQ ID NO: 37 - protein, 259 aa, Artificial Sequence
  CD34 ectodomain
SLDNNGTATPELPTQGTFSNVSTNVSYQETTTPSTLGSTSLHPVSQHGNEATTNITETTVKFTSTSVITSVYGNTNSSVQSQTSVISTVFTTPANVSTPETTLKPSLSPGNVSDLSTTSTSLATSPTKPYTSSSPILSDIKAEIKCSGIREVKLTQGICLEQNKTSSCAEFKKDRGEGLARVLCGEEQADADAGAQVCSLLLAQSEVRPQCLLLVLANRTEISSKLQLMKKHQSDLKKLGILDFTEQDVASHQSYSQKT

SEQ ID NO: 38 - protein, 27 aa, Artificial Sequence
  CD28 transmembrane domain
FWVLVVVGGVLACYSLLVTVAFIIFWV

SEQ ID NO: 39 - protein, 112 aa, Artificial Sequence
  CD3 Z endodomain
RVKFSRSADAPAYQQGQNQLYNELNLGRREEYDVLDKRRGRDPEMGGKPRRKNPQEGLYNELQKDKMAEAYSEIGMKGERRRGKGHDGLYQGLSTATKDTYDALHMQALPPR

SEQ ID NO: 40 - protein, 37 aa, Artificial Sequence
  CD28 endodomain
KRSRLLHSDYMNMTPRRPGPTRKHYQPYAPPRDFAAY

SEQ ID NO: 41 - protein, 37 aa, Artificial Sequence
  OX40 endodomain
RRDQRLPPDAHKPPGGGSFRTPIQEEQADAHSTLAKI

SEQ ID NO: 42 - protein, 42 aa, Artificial Sequence
  41BB endodomain
KRGRKKLLYIFKQPFMRPVQTTQEEDGCSCRFPEEEEGGCEL

SEQ ID NO: 43 - protein, 152 aa, Artificial Sequence
  CD28 and CD3 Zeta endodomains
SKRSRLLHSDYMNMTPRRPGPTRKHYQPYAPPRDFAAYRSRVKFSRSADAPAYQQGQNQLYNELNLGRREEYDVLDKRRGRDPEMGGKPRRKNPQEGLYNELQKDKMAEAYSEIGMKGERRRGKGHDGLYQGLSTATKDTYDALHMQALPPR

SEQ ID NO: 44 - protein, 188 aa, Artificial Sequence
  CD28, OX40 and CD3 Zeta endodomains
SKRSRLLHSDYMNMTPRRPGPTRKHYQPYAPPRDFAAYRSRDQRLPPDAHKPPGGGSFRTPIQEEQADAHSTLAKIRVKFSRSADAPAYQQGQNQLYNELNLGRREEYDVLDKRRGRDPEMGGKPRRKNPQEGLYNELQKDKMAEAYSEIGMKGERRRGKGHDGLYQGLSTATKDTYDALHMQALPPR

SEQ ID NO: 45 - protein, 191 aa, Artificial Sequence
  41BB, OX40 and CD3 Zeta endodomains
KRGRKKLLYIFKQPFMRPVQTTQEEDGCSCRFPEEEEGGCELRRDQRLPPDAHKPPGGGSFRTPIQEEQADAHSTLAKIRVKFSRSADAPAYQQGQNQLYNELNLGRREEYDVLDKRRGRDPEMGGKPRRKNPQEGLYNELQKDKMAEAYSEIGMKGERRRGKGHDGLYQGLSTATKDTYDALHMQALPPR

SEQ ID NO: 46 - protein, 20 aa, Foot-and-mouth disease virus
RAEGRGSLLTCGDVEENPGP

SEQ ID NO: 47 - protein, 20 aa, Foot-and-mouth disease virus
QCTNYALLKLAGDVESNPGP

SEQ ID NO: 48 - protein, 20 aa, Artificial Sequence
  cleavage site, 2A-like sequence
YHADYYKQRLIHDVEMNPGP

SEQ ID NO: 49 - protein, 20 aa, Artificial Sequence
  cleavage site, 2A-like sequence
HYAGYFADLLIHDIETNPGP

SEQ ID NO: 50 - protein, 20 aa, Artificial Sequence
  cleavage site, 2A-like sequence
QCTNYALLKLAGDVESNPGP

SEQ ID NO: 51 - protein, 19 aa, Artificial Sequence
  cleavage site, 2A-like sequence
ATNFSLLKQAGDVEENPGP

SEQ ID NO: 52 - protein, 19 aa, Artificial Sequence
  cleavage site, 2A-like sequence
AARQMLLLLSGDVETNPGP

SEQ ID NO: 53 - protein, 20 aa, Artificial Sequence
  cleavage site, 2A-like sequence
RAEGRGSLLTCGDVEENPGP

SEQ ID NO: 54 - protein, 20 aa, Artificial Sequence
  cleavage site, 2A-like sequence
TRAEIEDELIRAGIESNPGP

SEQ ID NO: 55 - protein, 20 aa, Artificial Sequence
  cleavage site, 2A-like sequence
TRAEIEDELIRADIESNPGP

SEQ ID NO: 56 - protein, 20 aa, Artificial Sequence
  cleavage site, 2A-like sequence
AKFQIDKILISGDVELNPGP

SEQ ID NO: 57 - protein, 20 aa, Artificial Sequence
  cleavage site, 2A-like sequence
SSIIRTKMLVSGDVEENPGP

SEQ ID NO: 58 - protein, 20 aa, Artificial Sequence
  cleavage site, 2A-like sequence
CDAQRQKLLLSGDIEQNPGP

SEQ ID NO: 59 - protein, 20 aa, Artificial Sequence
  cleavage site, 2A-like sequence
YPIDFGGFLVKADSEFNPGP

SEQ ID NO: 60 - DNA, 8736 bp, Artificial Sequence
  illustrative construct nucleic acid sequence
ggcctgaaataacctctgaaagaggaacttggttaggtaccttctgaggcggaaagaaccagctgtggaatgtgtgtcagttagggtgtggaaagtccccaggctccccagcaggcagaagtatgcaaagcatgcatctcaattagtcagcaaccaggtgtggaaagtccccaggctccccagcaggcagaagtatgcaaagcatgcatctcaattagtcagcaaccatagtcccttaagaatgtagtcttatgcaatactcttgtagtcttgcaacatggtaacgatgagttagcaacatgccttacaaggagagaaaaagcaccgtgcatgccgattggtggaagtaaggtggtacgatcgtgccttattaggaaggcaacagacgggtctgacatggattggacgaaccactgaattgccgcattgcagagatattgtatttaagtgcctagctcgatacaataaacgcgccagtcctccgattgactgcgtcgcccgggtacccgtattcccaataaagcctcttgctgtttgcatccgaatcgtggactcgctgatccttgggagggtctcctcagattgattgactgcccacctcgggggtctttcatttggaggttccaccgagatttggagacccctgcccagggaccaccgacccccccgccgggaggtaagctggccagcggtcgtttcgtgtctgtctctgtctttgggcgtgtttgtgccggcatctagtgtttgcgcctgcgtctgtactagttggctaactagatctgtatctggcggtcccgcggaagaactgacgagttcgtattcccggccgcagcccctgggagacgtcccagcggcctcgggggcccgttttgtggcccattctgtatcagttaacctacccgagtcggactttttggagctccgccactgtccgaggggtacgtggctttgttgggggacgagagacagagacacttcccgcccccgtctgaatttttgctttcggttttacgccgaaaccgcgccgcgcgtcttgtctgctgcagcatcgttctgtgttgtctctgtctgactgtgtttctgtatttgtctgaaaattagcggccgatctgacgcgactcgagtttactccctatcagtgatagagaacgtatgaagagtttactccctatcagtgatagagaacgtatgcagactttactccctatcagtgatagagaacgtataaggagtttactccctatcagtgatagagaacgtatgaccagtttactccctatcagtgatagagaacgtatctacagtttactccctatcagtgatagagaacgtatatccagtttactccctatcagtgatagagaacgtataagctttgcttatgtaaaccagggcgcctataaaagagtgctgattttttgagtaaacttcaattccacaacacttttgtcttataccaactttccgtaccacttcctaccctcgtaaagtcgacaccatggagaccgacaccctgctgctgtgggtgctgctgctgtgggtgccaggcagcaccggcgaggtgcagctgcagcagagcggacccgagctgatcaagccaggcgccagcgtgaagatgagctgcaaggccagcggctacaccttcaccagctacgtgatgcactgggtgaagcagaagccaggccagggcctggagtggatcggctacatcaacccctacaacgacggcaccaagtacaacgagaagttcaagggcaaggccaccctgaccagcgacaagagcagcagcaccgcctacatggagctgagcagcctgaccagcgaggacagcgccgtgtactactgcgccagaggcacctactactacggcagccgggtgttcgactactggggccagggcaccaccctgaccgtgagctctggcggaggcggctctggcggaggcggctctggcggaggcggcagcgacatcgtgatgacccaggctgcccccagcatccccgtgaccccaggcgagagcgtgagcatcagctgccggagcagcaagagcctgctgaacagcaacggcaacacctacctgtactggttcctgcagcggccaggccagagcccccagctgctgatctaccggatgagcaacctggccagcggcgtgcccgaccggttcagcggcagcggcagcggcaccgccttcaccctgcggatcagccgggtggaggccgaggacgtgggcgtgtactactgcatgcagcacctggagtaccccttcaccttcggagccggcaccaagctggagctgaagcggtcggatcccaccaccaccccagccccacggccacctacccctgccccaaccatcgccagccagcccctgagcctgcggcctgaagcctgcaggcctgccgccggaggagccgtgcacacaaggggcctggacttcgcctgcgacatctatatctgggcccccctggccgggacatgcggggtgctgctgctgtccctggtgattacactgtattgcaaacggggccggaagaagctgctgtacatcttcaagcagcccttcatgcggcccgtgcagaccacccaggaggaggacggctgcagctgccggttccccgaggaagaggaaggcggctgcgagctgcgggtgaagttcagccggagcgccgacgccccagcctaccagcagggccagaaccagctgtacaacgagctgaacctgggacggcgggaggagtacgacgtgctggacaagcggcggggacgggaccccgagatgggcggcaagcctcgccggaagaatccccaggagggcctgtacaacgagctgcagaaggacaagatggccgaggcctacagcgagatcggcatgaagggcgagcggcgccggggcaagggccacgacggcctgtaccagggcctgagcaccgccaccaaggacacctacgacgccctgcacatgcaggccctgccaccccggtgaacgcgtgccgctccggattagtccaatttgttaaagacaggattcgaggagcttgataattccacggggttggggttgcgccttttccaaggcagccctgggtttgcgcagggacgcggctgctctgggcgtggttccgggaaacgcagcggcgccgaccctgggtctcgcacattcttcacgtccgttcgcagcgtcacccggatcttcgccgctacccttgtgggccccccggcgacgcttcctgctccgcccctaagtcgggaaggttccttgcggttcgcggcgtgccggacgtgacaaacggaagccgcacgtctcactagtaccctcgcagacggacagcgccagggagcaatggcagcgcgccgaccgcgatgggctgtggccaatagcggctgctcagcagggcgcgccgagagcagcggccgggaaggggcggtgcgggaggcggggtgtggggcggtagtgtgggccctgttcctgcccgcgcggtgttccgcattctgcaagcctccggagcgcacgtcggcagtcggctccctcgttgaccgaatcaccgacctctctccccagggggatcatcgaattcgccaacatgcggccgcgccaccatgaagacgatcatcgccctgagctacatcttctgcctggtattcgccgactacaaggacgatgatgacgccagcatcgatatgtataatggctcctgttgccggattgaaggcgacactatctctcaagtaatgccccccctcctgatagtggccttcgtcctgggcgctcttggtaatggggttgcactctgtggtttctgtttccacatgaaaacctggaagccctcaacagtgtacctctttaaccttgccgtggcagacttcctgcttatgatttgcctgccctttaggaccgactattatctgcgacgccgccattgggctttcggcgacatcccctgtcgggttggtctgtttactctggctatgaatcgggccggcagtatcgtctttctcactgtggtcgctgccgacagatacttcaaggtagtgcacccccaccacgcagtgaacacaatctccactagagttgcagctggaattgtgtgcaccctgtgggctctggtaatcctgggcacagtatacctgctcctggagaatcatttgtgcgtgcaggagactgctgtgtcatgtgaatcttttattatggagtccgcaaacgggtggcatgatatcatgtttcaactggagttctttatgccccttggcatcattctgttttgctcattcaagatcgtttggtctctccggcgccggcagcagctggcccggcaagctcggatgaaaaaggccacgcgctttatcatggttgtggctatcgtcttcatcacctgctaccttccttccgtgtccgcaagactgtattttctgtggaccgtccccagcagcgcttgcgatcccagtgtccacggcgccctccacatcaccttgagctttacgtacatgaactctatgctggaccccctggtgtactattttagctctccctccttcccgaaattctataataaacttaagatctgcagcctcaaaccaaagcaaccaggccattccaagactcagcgccctgaagagatgcccattagcaaccttggtagacggagctgcatctccgtcgcgaactcatttcagtctcagtccgacggacagtgggacccacacattgttgagtggcacatcgataccggtggacgcaccccacccagcctgggtccccaagatgagtcctgcaccaccgccagctcctccctggccaaggacacttcatcgaccggtgagaacctgtacttccagctaagattagataaaagtaaagtgattaacagcgcattagagctgcttaatgaggtcggaatcgaaggtttaacaacccgtaaactcgcccagaagctaggtgtagagcagcctacattgtattggcatgtaaaaaataagcgggctttgctcgacgccttagccattgagatgttagataggcaccatactcacttttgccctttagaaggggaaagctggcaagattttttacgtaataacgctaaaagttttagatgtgctttactaagtcatcgcgatggagcaaaagtacatttaggtacacggcctacagaaaaacagtatgaaactctcgaaaatcaattagcctttttatgccaacaaggtttttcactagagaatgcattatatgcactcagcgctgtggggcattttactttaggttgcgtattggaagatcaagagcatcaagtcgctaaagaagaaagggaaacacctactactgatagtatgccgccattattacgacaagctatcgaattatttgatcaccaaggtgcagagccagccttcttattcggccttgaattgatcatatgcggattagaaaaacaacttaaatgtgaaagtgggtccgcgtacagccgcgcgcgtacgaaaaacaattacgggtctaccatcgagggcctgctcgatctcccggacgacgacgcccccgaagaggcggggctggcggctccgcgcctgtcctttctccccgcgggacacacgcgcagactgtcgacggcccccccgaccgatgtcagcctgggggacgagctccacttagacggcgaggacgtggcgatggcgcatgccgacgcgctagacgatttcgatctggacatgttgggggacggggattccccgggtccgggatttaccccccacgactccgccccctacggcgctctggatatggccgacttcgagtttgagcagatgtttaccgatgcccttggaattgacgagtacggtgggcagtgtactaattatgctctcttgaaattggctggagatgtcgagtccaaccctgggccaatgggtgaaaagccaggtaccagggtcttcaagaagtcgagccctaactgcaagctcaccgtgtacttgggcaagcgggacttcgtagatcacctggacaaagtggaccctgtagatggcgtggtgcttgtggaccctgactacctgaaggaccgcaaagtgtttgtgaccctcacctgcgccttccgctatggccgtgaagacctggatgtgctgggcttgtccttccgcaaagacctgttcatcgccacctaccaggccttccccccggtgcccaacccaccccggccccccacccgcctgcaggaccggctgctgaggaagctgggccagcatgcccaccccttcttcttcaccataccccagaatcttccatgctccgtcacactgcagccaggcccagaggatacaggaaaggcctgcggcgtagactttgagattcgagccttctgtgctaaatcactagaagagaaaagccacaaaaggaactctgtgcggctggtgatccgaaaggtgcagttcgccccggagaaacccggcccccagccttcagccgaaaccacacgccacttcctcatgtctgaccgctccctgcacctcgaggcttccctggacaaggagctgtactaccacggggagcccctcaatgtaaatgtccacgtcaccaacaactccaccaagaccgtcaagaagatcaaagtctctgtgagacagtacgccgacatctgcctcttcagcaccgcccagtacaagtgtcctgtggctcaactcgaacaagatgaccaggtatctcccagctccacattctgtaaggtgtacaccataaccccactgctcagtgacaaccgggagaagcggggtctcgccctggatgggaaactcaagcacgaggacaccaacctggcttccagcaccatcgtgaaggagggtgccaacaaggaggtgctgggaatcctggtgtcctacagggtcaaggtgaagctggtggtgtctcgaggcggggatgtctctgtggagctgccttttgttcttatgcaccccaagccccacgaccacatccccctccccagaccccagtcagccgctccggagacagatgtccctgtggacaccaacctcattgaatttgataccaactatgccacagatgatgacattgtgtttgaggactttgcccggcttcggctgaaggggatgaaggatgacgactatgatgatcaactctgcagcttgtttaagggaccacgtgattacaacccgatatcgagcaccatttgtcatttgacgaatgaatctgatgggcacacaacatcgttgtatggtattggatttggtcccttcatcattacaaacaagcacttgtttagaagaaataatggaacactgttggtccaatcactacatggtgtattcaaggtcaagaacaccacgactttgcaacaacacctcattgatgggagggacatgataattattcgcatgcctaaggatttcccaccatttcctcaaaagctgaaatttagagagccacaaagggaagagcgcatatgtcttgtgacaaccaacttccaaactaagagcatgtctagcatggtgtcagacactagttgcacattcccttcatctgatggcatattctggaagcattggattcaaaccaaggatgggcagtgtggcagtccattagtatcaactagagatgggttcattgttggtatacactcagcatcgaatttcaccaacacaaacaattatttcacaagcgtgccgaaaaacttcatggaattgttgacaaatcaggaggcgcagcagtgggttagtggttggcgattaaatgctgactcagtattgtgggggggccataaagttttcatgagcaaacctgaagagccttttcagccagttaaggaagcgactcaactcatgaatgaattggtgtactcgcaatgaggatcccccgggctgcaggaattcgagcatcttaccgccatttatacccatatttgttctgtttttcttgatttgggtatacatttaaatgttaataaaacaaaatggtggggcaatcatttacatttttagggatatgtaattactagttcaggtgtattgccacaagacaaacatgttaagaaactttcccgttatttacgctctgttcctgttaatcaacctctggattacaaaatttgtgaaagattgactgatattcttaactatgttgctccttttacgctgtgtggatatgctgctttaatgcctctgtatcatgctattgcttcccgtacggctttcgttttctcctccttgtataaatcctggttgctgtctctttatgaggagttgtggcccgttgtccgtcaacgtggcgtggtgtgctctgtgtttgctgacgcaacccccactggctggggcattgccaccacctgtcaactcctttctgggactttcgctttccccctcccgatcgccacggcagaactcatcgccgcctgccttgcccgctgctggacaggggctaggttgctgggcactgataattccgtggtgttgtcggggaagctgacgtcctttcgaattcgatatcaagcttaacacgagccatagatagaataaaagattttatttagtctccagaaaaaggggggaatgaaagaccccaccgctagcgatatcgaattcacaacccctcactcggcgcgccagtcctccgacagactgagtcgcccgggtacccgtgttctcaataaaccctcttgcagttgcatccgactcgtggtctcgctgttccttgggagggtctcctctgagtgattgactgcccacctcgggggtctt

SEQ ID NO: 61 - DNA, 11238 bp, Artificial Sequence
  illustrative construct nucleic acid sequence
ggcctgaaataacctctgaaagaggaacttggttaggtaccttctgaggcggaaagaaccagctgtggaatgtgtgtcagttagggtgtggaaagtccccaggctccccagcaggcagaagtatgcaaagcatgcatctcaattagtcagcaaccaggtgtggaaagtccccaggctccccagcaggcagaagtatgcaaagcatgcatctcaattagtcagcaaccatagtcccttaagaatgtagtcttatgcaatactcttgtagtcttgcaacatggtaacgatgagttagcaacatgccttacaaggagagaaaaagcaccgtgcatgccgattggtggaagtaaggtggtacgatcgtgccttattaggaaggcaacagacgggtctgacatggattggacgaaccactgaattgccgcattgcagagatattgtatttaagtgcctagctcgatacaataaacgcgccagtcctccgattgactgcgtcgcccgggtacccgtattcccaataaagcctcttgctgtttgcatccgaatcgtggactcgctgatccttgggagggtctcctcagattgattgactgcccacctcgggggtctttcatttggaggttccaccgagatttggagacccctgcccagggaccaccgacccccccgccgggaggtaagctggccagcggtcgtttcgtgtctgtctctgtctttgggcgtgtttgtgccggcatctagtgtttgcgcctgcgtctgtactagttggctaactagatctgtatctggcggtcccgcggaagaactgacgagttcgtattcccggccgcagcccctgggagacgtcccagcggcctcgggggcccgttttgtggcccattctgtatcagttaacctacccgagtcggactttttggagctccgccactgtccgaggggtacgtggctttgttgggggacgagagacagagacacttcccgcccccgtctgaatttttgctttcggttttacgccgaaaccgcgccgcgcgtcttgtctgctgcagcatcgttctgtgttgtctctgtctgactgtgtttctgtatttgtctgaaaattagcggccgatctgacgcgactcgagtttactccctatcagtgatagagaacgtatgaagagtttactccctatcagtgatagagaacgtatgcagactttactccctatcagtgatagagaacgtataaggagtttactccctatcagtgatagagaacgtatgaccagtttactccctatcagtgatagagaacgtatctacagtttactccctatcagtgatagagaacgtatatccagtttactccctatcagtgatagagaacgtataagctttgcttatgtaaaccagggcgcctataaaagagtgctgattttttgagtaaacttcaattccacaacacttttgtcttataccaactttccgtaccacttcctaccctcgtaaagtcgacaccatggagaccgacaccctgctgctgtgggtgctgctgctgtgggtgccaggcagcaccggcgaggtgcagctgcagcagagcggacccgagctgatcaagccaggcgccagcgtgaagatgagctgcaaggccagcggctacaccttcaccagctacgtgatgcactgggtgaagcagaagccaggccagggcctggagtggatcggctacatcaacccctacaacgacggcaccaagtacaacgagaagttcaagggcaaggccaccctgaccagcgacaagagcagcagcaccgcctacatggagctgagcagcctgaccagcgaggacagcgccgtgtactactgcgccagaggcacctactactacggcagccgggtgttcgactactggggccagggcaccaccctgaccgtgagctctggcggaggcggctctggcggaggcggctctggcggaggcggcagcgacatcgtgatgacccaggctgcccccagcatccccgtgaccccaggcgagagcgtgagcatcagctgccggagcagcaagagcctgctgaacagcaacggcaacacctacctgtactggttcctgcagcggccaggccagagcccccagctgctgatctaccggatgagcaacctggccagcggcgtgcccgaccggttcagcggcagcggcagcggcaccgccttcaccctgcggatcagccgggtggaggccgaggacgtgggcgtgtactactgcatgcagcacctggagtaccccttcaccttcggagccggcaccaagctggagctgaagcggtcggatcccaccaccaccccagccccacggccacctacccctgccccaaccatcgccagccagcccctgagcctgcggcctgaagcctgcaggcctgccgccggaggagccgtgcacacaaggggcctggacttcgcctgcgacatctatatctgggcccccctggccgggacatgcggggtgctgctgctgtccctggtgattacactgtattgcaaacggggccggaagaagctgctgtacatcttcaagcagcccttcatgcggcccgtgcagaccacccaggaggaggacggctgcagctgccggttccccgaggaagaggaaggcggctgcgagctgcgggtgaagttcagccggagcgccgacgccccagcctaccagcagggccagaaccagctgtacaacgagctgaacctgggacggcgggaggagtacgacgtgctggacaagcggcggggacgggaccccgagatgggcggcaagcctcgccggaagaatccccaggagggcctgtacaacgagctgcagaaggacaagatggccgaggcctacagcgagatcggcatgaagggcgagcggcgccggggcaagggccacgacggcctgtaccagggcctgagcaccgccaccaaggacacctacgacgccctgcacatgcaggccctgccaccccggtgaacgcgtgccgctccggattagtccaatttgttaaagacaggattcgaggagcttgataattccacggggttggggttgcgccttttccaaggcagccctgggtttgcgcagggacgcggctgctctgggcgtggttccgggaaacgcagcggcgccgaccctgggtctcgcacattcttcacgtccgttcgcagcgtcacccggatcttcgccgctacccttgtgggccccccggcgacgcttcctgctccgcccctaagtcgggaaggttccttgcggttcgcggcgtgccggacgtgacaaacggaagccgcacgtctcactagtaccctcgcagacggacagcgccagggagcaatggcagcgcgccgaccgcgatgggctgtggccaatagcggctgctcagcagggcgcgccgagagcagcggccgggaaggggcggtgcgggaggcggggtgtggggcggtagtgtgggccctgttcctgcccgcgcggtgttccgcattctgcaagcctccggagcgcacgtcggcagtcggctccctcgttgaccgaatcaccgacctctctccccagggggatcatcgaattcgccaacatgcggccgcgccaccatgaagacgatcatcgccctgagctacatcttctgcctggtattcgccgactacaaggacgatgatgacgccagcatcgatatgtataatggctcctgttgccggattgaaggcgacactatctctcaagtaatgccccccctcctgatagtggccttcgtcctgggcgctcttggtaatggggttgcactctgtggtttctgtttccacatgaaaacctggaagccctcaacagtgtacctctttaaccttgccgtggcagacttcctgcttatgatttgcctgccctttaggaccgactattatctgcgacgccgccattgggctttcggcgacatcccctgtcgggttggtctgtttactctggctatgaatcgggccggcagtatcgtctttctcactgtggtcgctgccgacagatacttcaaggtagtgcacccccaccacgcagtgaacacaatctccactagagttgcagctggaattgtgtgcaccctgtgggctctggtaatcctgggcacagtatacctgctcctggagaatcatttgtgcgtgcaggagactgctgtgtcatgtgaatcttttattatggagtccgcaaacgggtggcatgatatcatgtttcaactggagttctttatgccccttggcatcattctgttttgctcattcaagatcgtttggtctctccggcgccggcagcagctggcccggcaagctcggatgaaaaaggccacgcgctttatcatggttgtggctatcgtcttcatcacctgctaccttccttccgtgtccgcaagactgtattttctgtggaccgtccccagcagcgcttgcgatcccagtgtccacggcgccctccacatcaccttgagctttacgtacatgaactctatgctggaccccctggtgtactattttagctctccctccttcccgaaattctataataaacttaagatctgcagcctcaaaccaaagcaaccaggccattccaagactcagcgccctgaagagatgcccattagcaaccttggtagacggagctgcatctccgtcgcgaactcatttcagtctcagtccgacggacagtgggacccacacattgttgagtggcacatcgataccggtggacgcaccccacccagcctgggtccccaagatgagtcctgcaccaccgccagctcctccctggccaaggacacttcatcgaccggtgagaacctgtacttccagctaagattagataaaagtaaagtgattaacagcgcattagagctgcttaatgaggtcggaatcgaaggtttaacaacccgtaaactcgcccagaagctaggtgtagagcagcctacattgtattggcatgtaaaaaataagcgggctttgctcgacgccttagccattgagatgttagataggcaccatactcacttttgccctttagaaggggaaagctggcaagattttttacgtaataacgctaaaagttttagatgtgctttactaagtcatcgcgatggagcaaaagtacatttaggtacacggcctacagaaaaacagtatgaaactctcgaaaatcaattagcctttttatgccaacaaggtttttcactagagaatgcattatatgcactcagcgctgtggggcattttactttaggttgcgtattggaagatcaagagcatcaagtcgctaaagaagaaagggaaacacctactactgatagtatgccgccattattacgacaagctatcgaattatttgatcaccaaggtgcagagccagccttcttattcggccttgaattgatcatatgcggattagaaaaacaacttaaatgtgaaagtgggtccatggaaaccgtgattaaagtgattagcagcgcgccggtggtggcgatgccggtggtgattaaaaccgaaggcccggcgtggaccccgctggaaccggaagatacccgctggctggatggcaaacataaacgcaaaagcagccagtgcctggtgaaaagcagcatgagcggctatattccgagctgcctggataaagatgaacagtgcgtggtgtgcggcgataaaccgaccggctatcattatcgctgcattacctgcgaaggctgcaaaagcttttttcgccgcaccattcagaaaaacctgcatccgacctatagctgcacctatgatggctgctgcgtgattgataaaattacccgcaaccagtgccagctgtgccgctttaaaaaatgcattagcgtgggcatggcgatggatctggtgctggatgatagcaaacgcgtggcgaaacgcaaactgattgaagaaaaccgcgaacgccgccgcaaagaagaaatgattaaaagcctgcagcatcgcccgagcccgagcgcggaagaatgggaactgattcatgtggtgaccgaagcgcatcgcagcaccaacgcgcagggcagccattggaaacagcgccgcaaatttctgctggaagatattggccagagcccgatggcgagcatgctggatggcgataaagtggatctggaagcgtttaccgaatttaccaaaattattaccccggcgattacccgcgtggtggattttgcgaaaaacctgccgatgtttagcgaactgccgtgcgaagatcagattattctgctgaaaggctgctgcatggaaattatgagcctgcgcgcggcggtgcgctatgatccggaaagcgaaaccctgaccctgagcggcgaaatggcggtgaaacgcgaacagctgaaaaacggcggcctgggcgtggtgagcgatgcgatttttgatctgggcaaaagcctgagcgcgtttaacctggatgataccgaagtggcgctgctgcaggcggtgctgctgatgagcagcgatcgcaccggcctgatttgcgtggataaaattgaaaaatgccaggaaagctatctgctggcgtttgaacattatattaactatcgcaaacataacattccgcatttttggagcaaactgctgatgaaagtggcggatctgcgcatgattggcgcgtatcatgcgagccgctttctgcatatgaaagtggaatgcccgaccgaactgagcccgcaggaagtgggcccggatcattgcatgaaatgcgcgcattttattgatggcccgcattgcgtgaaagcgtgcccggcgggcgtgctgggcgaaaacgataccctggtgtggaaatatgcggatgcgaacgcggtgtgccagctgtgccatccgaactgcacccgcggctgcaaaggcccgggcctggaaggctgcccgaacggcagcaaaaccccgagcattgcggcgggcgtggtgggcggcctgctgtgcctggtggtggtgggcctgggcattggcctgtatctgcgccgccgccatattgtgcgcaaacgcaccctgcgccgcctgctgcaggaacgcgaactggtggaaccgctgaccccgagcggcgaagcgccgaaccaggcgcatctgcgcattctgaaagaaaccgaatttaaaaaagtgaaagtgctgggctttggcgcgtttggcaccgtgtataaaggcctgtggattccggaaggcgaaaaagtgaccattccggtggcgattaaagaactgcgcgaagcgaccagcccgaaagcgaacaaagaaattctggatgaagcgtatgtgatggcgagcgtggataacccgcatgtgtgccgcctgctgggcatttgcctgaccagcaccgtgcagctgattacccagctgatgccgtatggctgcctgctggattatattcgcgaacataaagataacattggcagccagtatctgctgaactggtgcgtgcagattgcgaaaggcatgaactatctggaagaacgccatatggtgcatcgcgatctggcggcgcgcaacgtgctggtgaaaaccccgcagcatgtgaaaattaccgattttggcctggcgaaacagctgggcgcggatgaaaaagaatatcatgcggaaggcggcaaagtgccgattaaatggatggcgctggaaagcattctgcatcgcatttatacccatcagagcgatgtgtggagctatggcgtgaccgtgtgggaactgatgacctttggcagcaaaccgtatgatggcattccggcgagcgaaattagcagcgtgctggaaaaaggcgaacgcctgccgcagccgccgatttgcaccattgatgtgtatatgattatggtgaaatgctggatgagcggcgcggatagccgcccgaaatttcgcgaactgattgcggaatttagcaaaatggcgcgcgatccgccgcgctatctggtgattcagggcgatgaacgcatgcatctgccgagcccgaccgatagcaaattttatcgcaccctgatggaagaagaagatatggaagatattgtggatgcggatgaatatctggtgccgcatcagggcttttttaacagcccgagcaccagccgcaccccgctgctgagcagcctgagcgcgaccagcaacaacagcgcgaccaaatgcattgatcgcaacggcggccatccggtgcgcgaagatggctttctgccggcgccggaatatgtgaaccagctgatgccgaaaaaaccgagcaccgcgatggtgcagaaccagatttataactatattagcctgaccgcgattagcaaactgccgatggatagccgctatcagaacagccatagcaccgcggtggataacccggaatatctggaacagtgtactaattatgctctcttgaaattggctggagatgtcgagtccaaccctgggccaatgggtgaaaagccaggtaccagggtcttcaagaagtcgagccctaactgcaagctcaccgtgtacttgggcaagcgggacttcgtagatcacctggacaaagtggaccctgtagatggcgtggtgcttgtggaccctgactacctgaaggaccgcaaagtgtttgtgaccctcacctgcgccttccgctatggccgtgaagacctggatgtgctgggcttgtccttccgcaaagacctgttcatcgccacctaccaggccttccccccggtgcccaacccaccccggccccccacccgcctgcaggaccggctgctgaggaagctgggccagcatgcccaccccttcttcttcaccataccccagaatcttccatgctccgtcacactgcagccaggcccagaggatacaggaaaggcctgcggcgtagactttgagattcgagccttctgtgctaaatcactagaagagaaaagccacaaaaggaactctgtgcggctggtgatccgaaaggtgcagttcgccccggagaaacccggcccccagccttcagccgaaaccacacgccacttcctcatgtctgaccgctccctgcacctcgaggcttccctggacaaggagctgtactaccacggggagcccctcaatgtaaatgtccacgtcaccaacaactccaccaagaccgtcaagaagatcaaagtctctgtgagacagtacgccgacatctgcctcttcagcaccgcccagtacaagtgtcctgtggctcaactcgaacaagatgaccaggtatctcccagctccacattctgtaaggtgtacaccataaccccactgctcagtgacaaccgggagaagcggggtctcgccctggatgggaaactcaagcacgaggacaccaacctggcttccagcaccatcgtgaaggagggtgccaacaaggaggtgctgggaatcctggtgtcctacagggtcaaggtgaagctggtggtgtctcgaggcggggatgtctctgtggagctgccttttgttcttatgcaccccaagccccacgaccacatccccctccccagaccccagtcagccgctccggagacagatgtccctgtggacaccaacctcattgaatttgataccaactatgccacagatgatgacattgtgtttgaggactttgcccggcttcggctgaaggggatgaaggatgacgactatgatgatcaactctgcagcttgtttaagggaccacgtgattacaacccgatatcgagcaccatttgtcatttgacgaatgaatctgatgggcacacaacatcgttgtatggtattggatttggtcccttcatcattacaaacaagcacttgtttagaagaaataatggaacactgttggtccaatcactacatggtgtattcaaggtcaagaacaccacgactttgcaacaacacctcattgatgggagggacatgataattattcgcatgcctaaggatttcccaccatttcctcaaaagctgaaatttagagagccacaaagggaagagcgcatatgtcttgtgacaaccaacttccaaactaagagcatgtctagcatggtgtcagacactagttgcacattcccttcatctgatggcatattctggaagcattggattcaaaccaaggatgggcagtgtggcagtccattagtatcaactagagatgggttcattgttggtatacactcagcatcgaatttcaccaacacaaacaattatttcacaagcgtgccgaaaaacttcatggaattgttgacaaatcaggaggcgcagcagtgggttagtggttggcgattaaatgctgactcagtattgtgggggggccataaagttttcatgagcaaacctgaagagccttttcagccagttaaggaagcgactcaactcatgaatgaattggtgtactcgcaatgaggatcccccgggctgcaggaattcgagcatcttaccgccatttatacccatatttgttctgtttttcttgatttgggtatacatttaaatgttaataaaacaaaatggtggggcaatcatttacatttttagggatatgtaattactagttcaggtgtattgccacaagacaaacatgttaagaaactttcccgttatttacgctctgttcctgttaatcaacctctggattacaaaatttgtgaaagattgactgatattcttaactatgttgctccttttacgctgtgtggatatgctgctttaatgcctctgtatcatgctattgcttcccgtacggctttcgttttctcctccttgtataaatcctggttgctgtctctttatgaggagttgtggcccgttgtccgtcaacgtggcgtggtgtgctctgtgtttgctgacgcaacccccactggctggggcattgccaccacctgtcaactcctttctgggactttcgctttccccctcccgatcgccacggcagaactcatcgccgcctgccttgcccgctgctggacaggggctaggttgctgggcactgataattccgtggtgttgtcggggaagctgacgtcctttcgaattcgatatcaagcttaacacgagccatagatagaataaaagattttatttagtctccagaaaaaggggggaatgaaagaccccaccgctagcgatatcgaattcacaacccctcactcggcgcgccagtcctccgacagactgagtcgcccgggtacccgtgttctcaataaaccctcttgcagttgcatccgactcgtggtctcgctgttccttgggagggtctcctctgagtgattgactgcccacctcgggggtctt